European Patent Specification EP 3 715 470 B1, published October 11, 2023. Title: PROBES FOR IMPROVED MELT DISCRIMINATION AND MULTIPLEXING IN NUCLEIC ACID ASSAYS. Applicant: Luminex Corporation. The sequence listing filed with the application follows.

SEQUENCE LISTING (21 sequences)

SEQ ID NO: 1 - DNA, 25 bp, Artificial sequence
  Synthetic probe
gaccaccgccattattacgaaccat

SEQ ID NO: 2 - DNA, 26 bp, Artificial sequence
  Synthetic probe
gaccaccgccattattacgaaccatc

SEQ ID NO: 3 - DNA, 27 bp, Artificial sequence
  Synthetic probe
gaccaccgccattattacgaaccatca

SEQ ID NO: 4 - DNA, 28 bp, Artificial sequence
  Synthetic probe
gaccaccgccattattacgaaccatcac

SEQ ID NO: 5 - DNA, 29 bp, Artificial sequence
  Synthetic probe
gaccaccgccattattacgaaccatcacg

SEQ ID NO: 6 - DNA, 30 bp, Artificial sequence
  Synthetic probe
gaccaccgccattattacgaaccatcacga

SEQ ID NO: 7 - DNA, 31 bp, Artificial sequence
  Synthetic probe
gaccaccgccattattacgaaccatcacgac

SEQ ID NO: 8 - DNA, 46 bp, Artificial sequence
  Synthetic probe
tcactcgagtcgtcgtgatgagctgtttgaatattagatggcacac

SEQ ID NO: 9 - DNA, 21 bp, Staphylococcus epidermidis
tcagcagttgaagggacagat

SEQ ID NO: 10 - DNA, 22 bp, Staphylococcus epidermidis
ccagaacaatgaatggttaagg

SEQ ID NO: 11 - DNA, 44 bp, Artificial sequence
  Synthetic probe
tcactcgagtcgtcgtgatgagctgtttgaatattagatggcac

SEQ ID NO: 12 - DNA, 27 bp, Artificial sequence
  Synthetic probe
ccaccgccattattacgaaccatcacg

SEQ ID NO: 13 - DNA, 44 bp, Artificial sequence; identical to SEQ ID NO: 11
  Synthetic probe

SEQ ID NO: 14 - DNA, 27 bp, Artificial sequence
  Synthetic probe
ccaccgccattattacgaaccatcacg

SEQ ID NO: 15 - DNA, 27 bp, Artificial sequence
  Synthetic probe
ccaccgccattatttcgaaccatcacg

SEQ ID NO: 16 - DNA, 27 bp, Artificial sequence
  Synthetic probe
ccaccgccataattacgaaccatcacg

SEQ ID NO: 17 - DNA, 27 bp, Artificial sequence
  Synthetic probe
ccaccgccattattacgtaccatcacg

SEQ ID NO: 18 - DNA, 42 bp, Artificial sequence
  Synthetic probe
tctttctcaattgaccaccgccattattacgaaccatcacga

SEQ ID NO: 19 - DNA, 42 bp, Artificial sequence
  Synthetic probe
tctttctcatcggaccaccgccattattacgaaccatcacga

SEQ ID NO: 20 - DNA, 46 bp, Artificial sequence
  Synthetic probe
tctttctcaatttcgtgatgagctgtttgaatattagatggcacac

SEQ ID NO: 21 - DNA, 43 bp, Artificial sequence
  Synthetic probe
tctttctcatcgtgatgagctgtttgaatattagatggcacac